European Patent Application EP 4 592 315 A1, published July 30, 2025. Title: ANTIBODY AND USE THEREOF IN RESISTING TUMOR. Applicant: BIOTHEUS INC. Application CN. The sequence listing filed with the application follows.

SEQUENCE LISTING (50 sequences)

SEQ ID NO: 1 - protein, 120 aa, synthetic construct [sequence omitted]

SEQ ID NO: 2 - protein, 107 aa, synthetic construct [sequence omitted]

SEQ ID NO: 3 - protein, 119 aa, synthetic construct [sequence omitted]

SEQ ID NO: 4 - protein, 107 aa, synthetic construct [sequence omitted]

SEQ ID NO: 5 - protein, 120 aa, synthetic construct
EVQLVESGGGLVQPGGSLRLSCAASGFNIKDTYIHWVRQAPGKGLEWVARIYPTQGYTRYADSVKGRFTISADTSKNTAYLQMNSLRAEDTAVYYCSRWGGEGFYAMDYWGQGTLVTVSS

SEQ ID NO: 6 - protein, 107 aa, synthetic construct
DIQMTQSPSSLSASVGDRVTITCRASQSVQGAVAWYQQKPGKAPKLLIYSASFLYSGVPSRFSGSRSGTDFTLTISSLQPEDFATYYCQQHSTTPPTFGQGTKVEIK

SEQ ID NO: 7 - protein, 125 aa, synthetic construct
QVQLVESGGGVVQPGRSLRLSCAASGSTFSIVAMGWYRQAPGKQRELVASIITGDGDTNYADSVKGRFTISRDNSKNTMYLQMNSLKPEDTAVYYCYARTGYGSSELEGHEYDYWGQGTQVTVSS

SEQ ID NO: 8 - protein, 9 aa, synthetic construct
QQHSTTPPT

SEQ ID NO: 9 - protein, 107 aa, synthetic construct [sequence omitted]

SEQ ID NO: 10 - protein, 329 aa, synthetic construct
ASTKGPSVFPLAPSSKSTSGGTAALGCLVKDYFPEPVTVSWNSGALTSGVHTFPAVLQSSGLYSLSSVVTVPSSSLGTQTYICNVNHKPSNTKVDKKVEPKSCDKTHTCPPCPAPELLGGPSVFLFPPKPKDTLMISRTPEVTCVVVDVSHEDPEVKFNWYVDGVEVHNAKTKPREEQYNSTYRVVSVLTVLHQDWLNGKEYKCKVSNKALPAPIEKTISKAKGQPREPQVYTLPPSREEMTKNQVSLTCLVKGFYPSDIAVEWESNGQPENNYKTTPPVLDSDGSFFLYSKLTVDKSRWQQGNVFSCSVMHEALHNHYTQKSLSLSPG

SEQ ID NO: 11 - protein, 329 aa, synthetic construct
ASTKGPSVFPLAPSSKSTSGGTAALGCLVKDYFPEPVTVSWNSGALTSGVHTFPAVLQSSGLYSLSSVVTVPSSSLGTQTYICNVNHKPSNTKVDKKVEPKSCDKTHTCPPCPAPEAAGGPSVFLFPPKPKDTLMISRTPEVTCVVVDVSHEDPEVKFNWYVDGVEVHNAKTKPREEQYNSTYRVVSVLTVLHQDWLNGKEYKCKVSNKALPAPIEKTISKAKGQPREPQVYTLPPSREEMTKNQVSLTCLVKGFYPSDIAVEWESNGQPENNYKTTPPVLDSDGSFFLYSKLTVDKSRWQQGNVFSCSVMHEALHNHYTQKSLSLSPG

SEQ ID NO: 12 - protein, 329 aa, synthetic construct
ASTKGPSVFPLAPSSKSTSGGTAALGCLVKDYFPEPVTVSWNSGALTSGVHTFPAVLQSSGLYSLSSVVTVPSSSLGTQTYICNVNHKPSNTKVDKKVEPKSCDKTHTCPPCPAPELLGGPSVFLFPPKPKDTLMISRTPEVTCVVVDVSHEDPEVKFNWYVDGVEVHNAKTKPREEQYNSTYRVVSVLTVLHQDWLNGKEYKCKVSNKALPAPIEKTISKAKGQPREPQVYTLPPSRDELTKNQVSLTCLVKGFYPSDIAVEWESNGQPENNYKTTPPVLDSDGSFFLYSKLTVDKSRWQQGNVFSCSVMHEALHNHYTQKSLSLSPG

SEQ ID NO: 13 - protein, 329 aa, synthetic construct
ASTKGPSVFPLAPSSKSTSGGTAALGCQVEDYFPEPVTVSWNSGALTSGVHTFPAVLQSSGLYELSSVVTVPSSSLGTQTYICNVNHKPSNTKVDKKVEPKSCDKTHTCPPCPAPELLGGPSVFLFPPKPKDTLMISRTPEVTCVVVDVSHEDPEVKFNWYVDGVEVHNAKTKPREEQYNSTYRVVSVLTVLHQDWLNGKEYKCKVSNKALPAPIEKTISKAKGQPREPQVYTLPPCRDELTKNQVSLWCLVKGFYPSDIAVEWESNGQPENNYKTTPPVLDSDGSFFLYSKLTVDKSRWQQGNVFSCSVMHEALHNHYTQKSLSLSPG

SEQ ID NO: 14 - protein, 329 aa, synthetic construct
ASTKGPSVFPRAPSSKSTSGGTAALGCLVRDYFPEPVTVSWNSGALTSGVHTFPAVLQSSGLYSLSSVVTVPSSSLGTQTYICNVNHKPSNTKVDKKVEPKSCDKTHTCPPCPAPELLGGPSVFLFPPKPKDTLMISRTPEVTCVVVDVSHEDPEVKFNWYVDGVEVHNAKTKPREEQYNSTYRVVSVLTVLHQDWLNGKEYKCKVSNKALPAPIEKTISKAKGQPREPQVCTLPPSRDELTKNQVSLSCAVKGFYPSDIAVEWESNGQPENNYKTTPPVLDSDGSFFLVSKLTVDKSRWQQGNVFSCSVMHEALHNHYTQKSLSLSPG

SEQ ID NO: 15 - protein, 107 aa, synthetic construct
RTVAAPSVFIFPPSDEQLKSGRASVVCLLNNFYPREAKVQWKVDNALQSGNSQESVTEQDSKDSTYSLSSRLQLSKADYEKHKVYACEVTHQGLSSPVTKSFNRGEC

SEQ ID NO: 16 - protein, 107 aa, synthetic construct
RTVAAPSVFIFPPSDEELKSGTASVQCLLNNFYPREAKVQWKVDNALQSGNSQESVTEQDSKDSTYSLSSELTLSKADYEKHKVYACEVTHQGLSSPVTKSFNRGEC

SEQ ID NO: 17 - protein, 21 aa, synthetic construct
GGGGSGGGGSGGGGSGGGGSG

SEQ ID NO: 18 - protein, 20 aa, synthetic construct
GGGGAGGGGAGGGGAGGGGA

SEQ ID NO: 19 - protein, 224 aa, synthetic construct
THTCPPCPAPELLGGPSVFLFPPKPKDTLMISRTPEVTCVVVDVSHEDPEVKFNWYVDGVEVHNAKTKPREEQYNSTYRVVSVLTVLHQDWLNGKEYKCKVSNKALPAPIEKTISKAKGQPREPQVYTLPPSREEMTKNQVSLTCLVKGFYPSDIAVEWESNGQPENNYKTTPPVLDSDGSFFLYSKLTVDKSRWQQGNVFSCSVMHEALHNHYTQKSLSLSPG

SEQ ID NO: 20 - protein, 224 aa, synthetic construct
THTCPPCPAPEAAGGPSVFLFPPKPKDTLMISRTPEVTCVVVDVSHEDPEVKFNWYVDGVEVHNAKTKPREEQYNSTYRVVSVLTVLHQDWLNGKEYKCKVSNKALPAPIEKTISKAKGQPREPQVYTLPPSREEMTKNQVSLTCLVKGFYPSDIAVEWESNGQPENNYKTTPPVLDSDGSFFLYSKLTVDKSRWQQGNVFSCSVMHEALHNHYTQKSLSLSPG

SEQ ID NO: 21 - protein, 594 aa, synthetic construct
EVQLVESGGGLVQPGGSLRLSCAASGFNIKDTYIHWVRQAPGKGLEWVARIYPTNGYTRYADSVKGRFTISADTSKNTAYLQMNSLRAEDTAVYYCSRWGGDGFYAMDYWGQGTLVTVSSASTKGPSVFPLAPSSKSTSGGTAALGCLVKDYFPEPVTVSWNSGALTSGVHTFPAVLQSSGLYSLSSVVTVPSSSLGTQTYICNVNHKPSNTKVDKKVEPKSCDKTHTCPPCPAPELLGGPSVFLFPPKPKDTLMISRTPEVTCVVVDVSHEDPEVKFNWYVDGVEVHNAKTKPREEQYNSTYRVVSVLTVLHQDWLNGKEYKCKVSNKALPAPIEKTISKAKGQPREPQVYTLPPSREEMTKNQVSLTCLVKGFYPSDIAVEWESNGQPENNYKTTPPVLDSDGSFFLYSKLTVDKSRWQQGNVFSCSVMHEALHNHYTQKSLSLSPGGGGGAGGGGAGGGGAGGGGAQVQLVESGGGVVQPGRSLRLSCAASGSTFSIVAMGWYRQAPGKQRELVASIITGDGDTNYADSVKGRFTISRDNSKNTMYLQMNSLKPEDTAVYYCYARTGYGSSELEGHEYDYWGQGTQVTVSS

SEQ ID NO: 22 - protein, 214 aa, synthetic construct
DIQMTQSPSSLSASVGDRVTITCRASQDVNTAVAWYQQKPGKAPKLLIYSASFLYSGVPSRFSGSRSGTDFTLTISSLQPEDFATYYCQQHYTTPPTFGQGTKVEIKRTVAAPSVFIFPPSDEQLKSGTASVVCLLNNFYPREAKVQWKVDNALQSGNSQESVTEQDSKDSTYSLSSTLTLSKADYEKHKVYACEVTHQGLSSPVTKSFNRGEC

SEQ ID NO: 23 - protein, 594 aa, synthetic construct
EVQLVESGGGLVQPGGSLRLSCAASGFNIKDTYIHWVRQAPGKGLEWVARIYPTNGYTRYADSVKGRFTISADTSKNTAYLQMNSLRAEDTAVYYCSRWGGDGFYAMDYWGQGTLVTVSSASTKGPSVFPLAPSSKSTSGGTAALGCLVKDYFPEPVTVSWNSGALTSGVHTFPAVLQSSGLYSLSSVVTVPSSSLGTQTYICNVNHKPSNTKVDKKVEPKSCDKTHTCPPCPAPEAAGGPSVFLFPPKPKDTLMISRTPEVTCVVVDVSHEDPEVKFNWYVDGVEVHNAKTKPREEQYNSTYRVVSVLTVLHQDWLNGKEYKCKVSNKALPAPIEKTISKAKGQPREPQVYTLPPSREEMTKNQVSLTCLVKGFYPSDIAVEWESNGQPENNYKTTPPVLDSDGSFFLYSKLTVDKSRWQQGNVFSCSVMHEALHNHYTQKSLSLSPGGGGGAGGGGAGGGGAGGGGAQVQLVESGGGVVQPGRSLRLSCAASGSTFSIVAMGWYRQAPGKQRELVASIITGDGDTNYADSVKGRFTISRDNSKNTMYLQMNSLKPEDTAVYYCYARTGYGSSELEGHEYDYWGQGTQVTVSS

SEQ ID NO: 24 - protein, 214 aa, synthetic construct; identical to SEQ ID NO: 22

SEQ ID NO: 25 - protein, 593 aa, synthetic construct
EVQLVESGGGLVQPGGSLRLSCAASGFTFTDYTMDWVRQAPGKGLEWVADVNPNSGGSIYNQRFKGRFTLSVDRSKNTLYLQMNSLRAEDTAVYYCARNLGPSFYFDYWGQGTLVTVSSASTKGPSVFPLAPSSKSTSGGTAALGCLVKDYFPEPVTVSWNSGALTSGVHTFPAVLQSSGLYSLSSVVTVPSSSLGTQTYICNVNHKPSNTKVDKKVEPKSCDKTHTCPPCPAPELLGGPSVFLFPPKPKDTLMISRTPEVTCVVVDVSHEDPEVKFNWYVDGVEVHNAKTKPREEQYNSTYRVVSVLTVLHQDWLNGKEYKCKVSNKALPAPIEKTISKAKGQPREPQVYTLPPSRDELTKNQVSLTCLVKGFYPSDIAVEWESNGQPENNYKTTPPVLDSDGSFFLYSKLTVDKSRWQQGNVFSCSVMHEALHNHYTQKSLSLSPGGGGGAGGGGAGGGGAGGGGAQVQLVESGGGVVQPGRSLRLSCAASGSTFSIVAMGWYRQAPGKQRELVASIITGDGDTNYADSVKGRFTISRDNSKNTMYLQMNSLKPEDTAVYYCYARTGYGSSELEGHEYDYWGQGTQVTVSS

SEQ ID NO: 26 - protein, 214 aa, synthetic construct
DIQMTQSPSSLSASVGDRVTITCKASQDVSIGVAWYQQKPGKAPKLLIYSASYRYTGVPSRFSGSGSGTDFTLTISSLQPEDFATYYCQQYYIYPYTFGQGTKVEIKRTVAAPSVFIFPPSDEQLKSGTASVVCLLNNFYPREAKVQWKVDNALQSGNSQESVTEQDSKDSTYSLSSTLTLSKADYEKHKVYACEVTHQGLSSPVTKSFNRGEC

SEQ ID NO: 27 - protein, 594 aa, synthetic construct
EVQLVESGGGLVQPGGSLRLSCAASGFNIKDTYIHWVRQAPGKGLEWVARIYPTQGYTRYADSVKGRFTISADTSKNTAYLQMNSLRAEDTAVYYCSRWGGEGFYAMDYWGQGTLVTVSSASTKGPSVFPLAPSSKSTSGGTAALGCQVEDYFPEPVTVSWNSGALTSGVHTFPAVLQSSGLYELSSVVTVPSSSLGTQTYICNVNHKPSNTKVDKKVEPKSCDKTHTCPPCPAPELLGGPSVFLFPPKPKDTLMISRTPEVTCVVVDVSHEDPEVKFNWYVDGVEVHNAKTKPREEQYNSTYRVVSVLTVLHQDWLNGKEYKCKVSNKALPAPIEKTISKAKGQPREPQVYTLPPCRDELTKNQVSLWCLVKGFYPSDIAVEWESNGQPENNYKTTPPVLDSDGSFFLYSKLTVDKSRWQQGNVFSCSVMHEALHNHYTQKSLSLSPGGGGGAGGGGAGGGGAGGGGAQVQLVESGGGVVQPGRSLRLSCAASGSTFSIVAMGWYRQAPGKQRELVASIITGDGDTNYADSVKGRFTISRDNSKNTMYLQMNSLKPEDTAVYYCYARTGYGSSELEGHEYDYWGQGTQVTVSS

SEQ ID NO: 28 - protein, 214 aa, synthetic construct
DIQMTQSPSSLSASVGDRVTITCRASQSVQGAVAWYQQKPGKAPKLLIYSASFLYSGVPSRFSGSRSGTDFTLTISSLQPEDFATYYCQQHSTTPPTFGQGTKVEIKRTVAAPSVFIFPPSDEQLKSGRASVVCLLNNFYPREAKVQWKVDNALQSGNSQESVTEQDSKDSTYSLSSRLQLSKADYEKHKVYACEVTHQGLSSPVTKSFNRGEC

SEQ ID NO: 29 - protein, 593 aa, synthetic construct
EVQLVESGGGLVQPGGSLRLSCAASGFTFTDYTMDWVRQAPGKGLEWVADVNPNSGGSIYNQRFKGRFTLSVDRSKNTLYLQMNSLRAEDTAVYYCARNLGPSFYFDYWGQGTLVTVSSASTKGPSVFPRAPSSKSTSGGTAALGCLVRDYFPEPVTVSWNSGALTSGVHTFPAVLQSSGLYSLSSVVTVPSSSLGTQTYICNVNHKPSNTKVDKKVEPKSCDKTHTCPPCPAPELLGGPSVFLFPPKPKDTLMISRTPEVTCVVVDVSHEDPEVKFNWYVDGVEVHNAKTKPREEQYNSTYRVVSVLTVLHQDWLNGKEYKCKVSNKALPAPIEKTISKAKGQPREPQVCTLPPSRDELTKNQVSLSCAVKGFYPSDIAVEWESNGQPENNYKTTPPVLDSDGSFFLVSKLTVDKSRWQQGNVFSCSVMHEALHNHYTQKSLSLSPGGGGGAGGGGAGGGGAGGGGAQVQLVESGGGVVQPGRSLRLSCAASGSTFSIVAMGWYRQAPGKQRELVASIITGDGDTNYADSVKGRFTISRDNSKNTMYLQMNSLKPEDTAVYYCYARTGYGSSELEGHEYDYWGQGTQVTVSS

SEQ ID NO: 30 - protein, 214 aa, synthetic construct
DIQMTQSPSSLSASVGDRVTITCKASQDVSIGVAWYQQKPGKAPKLLIYSASYRYTGVPSRFSGSGSGTDFTLTISSLQPEDFATYYCQQYYIYPYTFGQGTKVEIKRTVAAPSVFIFPPSDEELKSGTASVQCLLNNFYPREAKVQWKVDNALQSGNSQESVTEQDSKDSTYSLSSELTLSKADYEKHKVYACEVTHQGLSSPVTKSFNRGEC

SEQ ID NO: 31 - protein, 370 aa, synthetic construct
THTCPPCPAPELLGGPSVFLFPPKPKDTLMISRTPEVTCVVVDVSHEDPEVKFNWYVDGVEVHNAKTKPREEQYNSTYRVVSVLTVLHQDWLNGKEYKCKVSNKALPAPIEKTISKAKGQPREPQVYTLPPSREEMTKNQVSLTCLVKGFYPSDIAVEWESNGQPENNYKTTPPVLDSDGSFFLYSKLTVDKSRWQQGNVFSCSVMHEALHNHYTQKSLSLSPGGGGGSGGGGSGGGGSGGGGSGQVQLVESGGGVVQPGRSLRLSCAASGSTFSIVAMGWYRQAPGKQRELVASIITGDGDTNYADSVKGRFTISRDNSKNTMYLQMNSLKPEDTAVYYCYARTGYGSSELEGHEYDYWGQGTQVTVSS

SEQ ID NO: 32 - protein, 370 aa, synthetic construct
THTCPPCPAPEAAGGPSVFLFPPKPKDTLMISRTPEVTCVVVDVSHEDPEVKFNWYVDGVEVHNAKTKPREEQYNSTYRVVSVLTVLHQDWLNGKEYKCKVSNKALPAPIEKTISKAKGQPREPQVYTLPPSREEMTKNQVSLTCLVKGFYPSDIAVEWESNGQPENNYKTTPPVLDSDGSFFLYSKLTVDKSRWQQGNVFSCSVMHEALHNHYTQKSLSLSPGGGGGSGGGGSGGGGSGGGGSGQVQLVESGGGVVQPGRSLRLSCAASGSTFSIVAMGWYRQAPGKQRELVASIITGDGDTNYADSVKGRFTISRDNSKNTMYLQMNSLKPEDTAVYYCYARTGYGSSELEGHEYDYWGQGTQVTVSS

SEQ ID NO: 33 - protein, 447 aa, synthetic construct
QVQLQQWGAGLLKPSETLSLTCAVYGGSFSGYYWSWIRQSPEKGLEWIGEINHGGYVTYNPSLESRVTISVDTSKNQFSLKLSSVTAADTAVYYCARDYGPGNYDWYFDLWGRGTLVTVSSASTKGPSVFPLAPCSRSTSESTAALGCLVKDYFPEPVTVSWNSGALTSGVHTFPAVLQSSGLYSLSSVVTVPSSSLGTKTYTCNVDHKPSNTKVDKRVESKYGPPCPPCPAPEFLGGPSVFLFPPKPKDTLMISRTPEVTCVVVDVSQEDPEVQFNWYVDGVEVHNAKTKPREEQFNSTYRVVSVLTVLHQDWLNGKEYKCKVSNKGLPSSIEKTISKAKGQPREPQVYTLPPSQEEMTKNQVSLTCLVKGFYPSDIAVEWESNGQPENNYKTTPPVLDSDGSFFLYSRLTVDKSRWQEGNVFSCSVMHEALHNHYTQKSLSLSLG

SEQ ID NO: 34 - protein, 216 aa, synthetic construct
EIVLTQSPATLSLSPGERATLSCRASQSVSSYLAWYQQKPGQAPRLLIYDASNRATGIPARFSGSGSGTDFTLTISSLEPEDFAVYYCQQRSNWPPALTFGGGTKVEIKRTVAAPSVFIFPPSDEQLKSGTASVVCLLNNFYPREAKVQWKVDNALQSGNSQESVTEQDSKDSTYSLSSTLTLSKADYEKHKVYACEVTHQGLSSPVTKSFNRGEC

SEQ ID NO: 35 - protein, 640 aa, synthetic construct
EVQLVESGGGLVQPGGSLRLSCAASGFNIKDTYIHWVRQAPGKGLEWVARIYPTNGYTRYADSVKGRFTISADTSKNTAYLQMNSLRAEDTAVYYCSRWGGDGFYAMDYWGQGTLVTVSSASTKGPSVFPLAPCSRSTSESTAALGCLVKDYFPEPVTVSWNSGALTSGVHTFPAVLQSSGLYSLSSVVTVPSSSLGTKTYTCNVDHKPSNTKVDKRVESKYGPPCPPCPAPEAAGGPSVFLFPPKPKDTLMISRTPEVTCVVVDVSQEDPEVQFNWYVDGVEVHNAKTKPREEQFNSTYRVVSVLTVLHQDWLNGKEYKCKVSNKGLPSSIEKTISKAKGQPREPQVYTLPPSQEEMTKNQVSLTCLVKGFYPSDIAVEWESNGQPENNYKTTPPVLDSDGSFFLYSRLTVDKSRWQEGNVFSCSVMHEALHNHYTQKSLSLSLGKGGGGSGGGGSGGGGSQDSTSDLIPAPPLSKVPLQQNFQDNQFHGKWYVVGQAGNIRLREDKDPIKMMATIYELKEDKSYDVTMVKFDDKKCMYDIWTFVPGSQPGEFTLGKIKSFPGHTSSLVRVVSTNYNQHAMVFFKFVFQNREEFYITLYGRTKELTSELKENFIRFSKSLGLPENHIVFPVPIDQCIDG

SEQ ID NO: 36 - protein, 214 aa, synthetic construct; identical to SEQ ID NO: 22

SEQ ID NO: 37 - protein, 329 aa, synthetic construct
ASTKGPSVFPLAPSSKSTSGGTAALGCLVKDYFPEPVTVSWNSGALTSGVHTFPAVLQSSGLYSLSSVVTVPSSSLGTQTYICNVNHKPSNTKVDKKVEPKSCDKTHTCPPCPAPELLGGPSVFLFPPKPKDTLMISRTPEVTCVVVDVSHEDPEVKFNWYVDGVEVHNAKTKPREEQYNSTYRVVSVLTVLHQDWLNGKEYKCKVSNKALPAPIEKTISKAKGQPREPQVYTEPPSRDELTKNQVSLTCLVKGFYPSDIAVEWESNGQPENNYKTTPPVLDSDGSFFLLSVLTVDKSRWQQGNVFSCSVMHEALHNHYTQKSLSLSPG

SEQ ID NO: 38 - protein, 329 aa, synthetic construct
ASTKGPSVFPLAPSSKSTSGGTAALGCLVKDYFPEPVTVSWNSGALTSGVHTFPAVLQSSGLYSLSSVVTVPSSSLGTQTYICNVNHKPSNTKVDKKVEPKSCDKTHTCPPCPAPELLGGPSVFLFPPKPKDTLMISRTPEVTCVVVDVSHEDPEVKFNWYVDGVEVHNAKTKPREEQYNSTYRVVSVLTVLHQDWLNGKEYKCKVSNKALPAPIEKTISKAKGQPREPQVYTLPPSRDELTKNQVSLLCLVKGFYPSDIAVEWESNGQPENNYKTTPPVLRSDGSFFLYSKLTVDKSRWQQGNVFSCSVMHEALHNHYTQKSLSLSPG

SEQ ID NO: 39 - protein, 594 aa, synthetic construct
EVQLVESGGGLVQPGGSLRLSCAASGFNIKDTYIHWVRQAPGKGLEWVARIYPTNGYTRYADSVKGRFTISADTSKNTAYLQMNSLRAEDTAVYYCSRWGGDGFYAMDYWGQGTLVTVSSASTKGPSVFPLAPSSKSTSGGTAALGCLVKDYFPEPVTVSWNSGALTSGVHTFPAVLQSSGLYSLSSVVTVPSSSLGTQTYICNVNHKPSNTKVDKKVEPKSCDKTHTCPPCPAPELLGGPSVFLFPPKPKDTLMISRTPEVTCVVVDVSHEDPEVKFNWYVDGVEVHNAKTKPREEQYNSTYRVVSVLTVLHQDWLNGKEYKCKVSNKALPAPIEKTISKAKGQPREPQVYTEPPSRDELTKNQVSLTCLVKGFYPSDIAVEWESNGQPENNYKTTPPVLDSDGSFFLLSVLTVDKSRWQQGNVFSCSVMHEALHNHYTQKSLSLSPGGGGGAGGGGAGGGGAGGGGAQVQLVESGGGVVQPGRSLRLSCAASGSTFSIVAMGWYRQAPGKQRELVASIITGDGDTNYADSVKGRFTISRDNSKNTMYLQMNSLKPEDTAVYYCYARTGYGSSELEGHEYDYWGQGTQVTVSS

SEQ ID NO: 40 - protein, 214 aa, synthetic construct; identical to SEQ ID NO: 22

SEQ ID NO: 41 - protein, 594 aa, synthetic construct
EVQLVESGGGLVQPGGSLRLSCAASGFTFTDYTMDWVRQAPGKGLEWVADVNPNSGGSIYNQRFKGRFTLSVDRSKNTLYLQMNSLRAEDTAVYYCARNLGPSFYFDYWGQGTLVTVSSASTKGPSVFPLAPSSKSTSGGTAALGCLVKDYFPEPVTVSWNSGALTSGVHTFPAVLQSSGLYSLSSVVTVPSSSLGTQTYICNVNHKPSNTKVDKKVEPKSCDKTHTCPPCPAPELLGGPSVFLFPPKPKDTLMISRTPEVTCVVVDVSHEDPEVKFNWYVDGVEVHNAKTKPREEQYNSTYRVVSVLTVLHQDWLNGKEYKCKVSNKALPAPIEKTISKAKGQPREPQVYTLPPSRDELTKNQVSLLCLVKGFYPSDIAVEWESNGQPENNYKTTPPVLRSDGSFFLYSKLTVDKSRWQQGNVFSCSVMHEALHNHYTQKSLSLSPGGGGGGAGGGGAGGGGAGGGGAQVQLVESGGGVVQPGRSLRLSCAASGSTFSIVAMGWYRQAPGKQRELVASIITGDGDTNYADSVKGRFTISRDNSKNTMYLQMNSLKPEDTAVYYCYARTGYGSSELEGHEYDYWGQGTQVTVSS

SEQ ID NO: 42 - protein, 214 aa, synthetic construct; identical to SEQ ID NO: 26

SEQ ID NO: 43 - protein, 8 aa, synthetic construct
GSTFSIVA

SEQ ID NO: 44 - protein, 8 aa, synthetic construct
IITGDGDT

SEQ ID NO: 45 - protein, 18 aa, synthetic construct
YARTGYGSSELEGHEYDY

SEQ ID NO: 46 - protein, 8 aa, synthetic construct
GFNIKDTY

SEQ ID NO: 47 - protein, 8 aa, synthetic construct
IYPTQGYT

SEQ ID NO: 48 - protein, 13 aa, synthetic construct
SRWGGEGFYAMDY

SEQ ID NO: 49 - protein, 6 aa, synthetic construct
QSVQGA

SEQ ID NO: 50 - skipped